European Patent Application EP 4 382 132 A1, published June 12, 2024. Title: Novel synthetic nucleic acid ligands and use thereof, and a pharmaceutical composition for alleviating or treating cancer comprising thereof as an active ingredient. Applicant: INTEROLIGO CORPORATION. Application WO. The sequence listing filed with the application follows.

SEQUENCE LISTING (23 sequences)

SEQ ID NO: 1 - DNA, 74 bp, synthetic construct
  source 1..74: mol_type = other DNA
  modified_base 19: mod_base = OTHER; note = 5-(N-(1-naphthylmethyl)carboxamide)-2'-deoxyuridine(Nap-dU)
  modified_base 21: mod_base = OTHER; note = 5-(N-(1-naphthylmethyl)carboxamide)-2'-deoxyuridine(Nap-dU)
  modified_base 28: mod_base = OTHER; note = 5-(N-(1-naphthylmethyl)carboxamide)-2'-deoxyuridine(Nap-dU)
  modified_base 34: mod_base = OTHER; note = 5-(N-(1-naphthylmethyl)carboxamide)-2'-deoxyuridine(Nap-dU)
  modified_base 36: mod_base = OTHER; note = 5-(N-(1-naphthylmethyl)carboxamide)-2'-deoxyuridine(Nap-dU)
  modified_base 42: mod_base = OTHER; note = 5-(N-(1-naphthylmethyl)carboxamide)-2'-deoxyuridine(Nap-dU)
  modified_base 44: mod_base = OTHER; note = 5-(N-(1-naphthylmethyl)carboxamide)-2'-deoxyuridine(Nap-dU)
  modified_base 46: mod_base = OTHER; note = 5-(N-(1-naphthylmethyl)carboxamide)-2'-deoxyuridine(Nap-dU)
  modified_base 51: mod_base = OTHER; note = 5-(N-(1-naphthylmethyl)carboxamide)-2'-deoxyuridine(Nap-dU)
  modified_base 56: mod_base = OTHER; note = 5-(N-(1-naphthylmethyl)carboxamide)-2'-deoxyuridine(Nap-dU)
gagtgaccgtctgcctgcncncccaggncgagcngnacgcgngngngaccngacgngcagccacaccaccagcc

SEQ ID NO: 2 - DNA, 50 bp, synthetic construct
  source 1..50: mol_type = other DNA
  modified_base 7: mod_base = OTHER; note = 5-(N-(1-naphthylmethyl)carboxamide)-2'-deoxyuridine(Nap-dU)
  modified_base 9: mod_base = OTHER; note = 5-(N-(1-naphthylmethyl)carboxamide)-2'-deoxyuridine(Nap-dU)
  modified_base 16: mod_base = OTHER; note = 5-(N-(1-naphthylmethyl)carboxamide)-2'-deoxyuridine(Nap-dU)
  modified_base 22: mod_base = OTHER; note = 5-(N-(1-naphthylmethyl)carboxamide)-2'-deoxyuridine(Nap-dU)
  modified_base 24: mod_base = OTHER; note = 5-(N-(1-naphthylmethyl)carboxamide)-2'-deoxyuridine(Nap-dU)
  modified_base 30: mod_base = OTHER; note = 5-(N-(1-naphthylmethyl)carboxamide)-2'-deoxyuridine(Nap-dU)
  modified_base 32: mod_base = OTHER; note = 5-(N-(1-naphthylmethyl)carboxamide)-2'-deoxyuridine(Nap-dU)
  modified_base 34: mod_base = OTHER; note = 5-(N-(1-naphthylmethyl)carboxamide)-2'-deoxyuridine(Nap-dU)
  modified_base 39: mod_base = OTHER; note = 5-(N-(1-naphthylmethyl)carboxamide)-2'-deoxyuridine(Nap-dU)
  modified_base 44: mod_base = OTHER; note = 5-(N-(1-naphthylmethyl)carboxamide)-2'-deoxyuridine(Nap-dU)
gcctgcncncccaggncgagcngnacgcgngngngaccngacgngcagcc

SEQ ID NO: 3 - DNA, 40 bp, synthetic construct
  source 1..40: mol_type = other DNA
  modified_base 2: mod_base = OTHER; note = 5-(N-(1-naphthylmethyl)carboxamide)-2'-deoxyuridine(Nap-dU)
  modified_base 4: mod_base = OTHER; note = 5-(N-(1-naphthylmethyl)carboxamide)-2'-deoxyuridine(Nap-dU)
  modified_base 11: mod_base = OTHER; note = 5-(N-(1-naphthylmethyl)carboxamide)-2'-deoxyuridine(Nap-dU)
  modified_base 17: mod_base = OTHER; note = 5-(N-(1-naphthylmethyl)carboxamide)-2'-deoxyuridine(Nap-dU)
  modified_base 19: mod_base = OTHER; note = 5-(N-(1-naphthylmethyl)carboxamide)-2'-deoxyuridine(Nap-dU)
  modified_base 25: mod_base = OTHER; note = 5-(N-(1-naphthylmethyl)carboxamide)-2'-deoxyuridine(Nap-dU)
  modified_base 27: mod_base = OTHER; note = 5-(N-(1-naphthylmethyl)carboxamide)-2'-deoxyuridine(Nap-dU)
  modified_base 29: mod_base = OTHER; note = 5-(N-(1-naphthylmethyl)carboxamide)-2'-deoxyuridine(Nap-dU)
  modified_base 34: mod_base = OTHER; note = 5-(N-(1-naphthylmethyl)carboxamide)-2'-deoxyuridine(Nap-dU)
  modified_base 39: mod_base = OTHER; note = 5-(N-(1-naphthylmethyl)carboxamide)-2'-deoxyuridine(Nap-dU)
cncncccaggncgagcngnacgcgngngngaccngacgng

SEQ ID NO: 4 - DNA, 35 bp, synthetic construct
  source 1..35: mol_type = other DNA
  modified_base 2: mod_base = OTHER; note = 5-(N-(1-naphthylmethyl)carboxamide)-2'-deoxyuridine(Nap-dU)
  modified_base 4: mod_base = OTHER; note = 5-(N-(1-naphthylmethyl)carboxamide)-2'-deoxyuridine(Nap-dU)
  modified_base 11: mod_base = OTHER; note = 5-(N-(1-naphthylmethyl)carboxamide)-2'-deoxyuridine(Nap-dU)
  modified_base 17: mod_base = OTHER; note = 5-(N-(1-naphthylmethyl)carboxamide)-2'-deoxyuridine(Nap-dU)
  modified_base 19: mod_base = OTHER; note = 5-(N-(1-naphthylmethyl)carboxamide)-2'-deoxyuridine(Nap-dU)
  modified_base 25: mod_base = OTHER; note = 5-(N-(1-naphthylmethyl)carboxamide)-2'-deoxyuridine(Nap-dU)
  modified_base 27: mod_base = OTHER; note = 5-(N-(1-naphthylmethyl)carboxamide)-2'-deoxyuridine(Nap-dU)
  modified_base 29: mod_base = OTHER; note = 5-(N-(1-naphthylmethyl)carboxamide)-2'-deoxyuridine(Nap-dU)
  modified_base 34: mod_base = OTHER; note = 5-(N-(1-naphthylmethyl)carboxamide)-2'-deoxyuridine(Nap-dU)
cncncccaggncgagcngnacgcgngngngaccng

SEQ ID NO: 5 - DNA, 35 bp, synthetic construct
  source 1..35: mol_type = other DNA
  modified_base 6: mod_base = OTHER; note = 5-(N-(1-naphthylmethyl)carboxamide)-2'-deoxyuridine(Nap-dU)
  modified_base 12: mod_base = OTHER; note = 5-(N-(1-naphthylmethyl)carboxamide)-2'-deoxyuridine(Nap-dU)
  modified_base 14: mod_base = OTHER; note = 5-(N-(1-naphthylmethyl)carboxamide)-2'-deoxyuridine(Nap-dU)
  modified_base 20: mod_base = OTHER; note = 5-(N-(1-naphthylmethyl)carboxamide)-2'-deoxyuridine(Nap-dU)
  modified_base 22: mod_base = OTHER; note = 5-(N-(1-naphthylmethyl)carboxamide)-2'-deoxyuridine(Nap-dU)
  modified_base 24: mod_base = OTHER; note = 5-(N-(1-naphthylmethyl)carboxamide)-2'-deoxyuridine(Nap-dU)
  modified_base 29: mod_base = OTHER; note = 5-(N-(1-naphthylmethyl)carboxamide)-2'-deoxyuridine(Nap-dU)
  modified_base 34: mod_base = OTHER; note = 5-(N-(1-naphthylmethyl)carboxamide)-2'-deoxyuridine(Nap-dU)
ccaggncgagcngnacgcgngngngaccngacgng

SEQ ID NO: 6 - DNA, 30 bp, synthetic construct
  source 1..30: mol_type = other DNA
  modified_base 1: mod_base = OTHER; note = 5-(N-(1-naphthylmethyl)carboxamide)-2'-deoxyuridine(Nap-dU)
  modified_base 8: mod_base = OTHER; note = 5-(N-(1-naphthylmethyl)carboxamide)-2'-deoxyuridine(Nap-dU)
  modified_base 14: mod_base = OTHER; note = 5-(N-(1-naphthylmethyl)carboxamide)-2'-deoxyuridine(Nap-dU)
  modified_base 16: mod_base = OTHER; note = 5-(N-(1-naphthylmethyl)carboxamide)-2'-deoxyuridine(Nap-dU)
  modified_base 22: mod_base = OTHER; note = 5-(N-(1-naphthylmethyl)carboxamide)-2'-deoxyuridine(Nap-dU)
  modified_base 24: mod_base = OTHER; note = 5-(N-(1-naphthylmethyl)carboxamide)-2'-deoxyuridine(Nap-dU)
  modified_base 26: mod_base = OTHER; note = 5-(N-(1-naphthylmethyl)carboxamide)-2'-deoxyuridine(Nap-dU)
ncccaggncgagcngnacgcgngngngacc

SEQ ID NO: 7 - DNA, 29 bp, synthetic construct
  source 1..29: mol_type = other DNA
  modified_base 5: mod_base = OTHER; note = 5-(N-(1-naphthylmethyl)carboxamide)-2'-deoxyuridine(Nap-dU)
  modified_base 11: mod_base = OTHER; note = 5-(N-(1-naphthylmethyl)carboxamide)-2'-deoxyuridine(Nap-dU)
  modified_base 13: mod_base = OTHER; note = 5-(N-(1-naphthylmethyl)carboxamide)-2'-deoxyuridine(Nap-dU)
  modified_base 19: mod_base = OTHER; note = 5-(N-(1-naphthylmethyl)carboxamide)-2'-deoxyuridine(Nap-dU)
  modified_base 21: mod_base = OTHER; note = 5-(N-(1-naphthylmethyl)carboxamide)-2'-deoxyuridine(Nap-dU)
  modified_base 23: mod_base = OTHER; note = 5-(N-(1-naphthylmethyl)carboxamide)-2'-deoxyuridine(Nap-dU)
  modified_base 28: mod_base = OTHER; note = 5-(N-(1-naphthylmethyl)carboxamide)-2'-deoxyuridine(Nap-dU)
caggncgagcngnacgcgngngngaccng

SEQ ID NO: 8 - DNA, 27 bp, synthetic construct
  source 1..27: mol_type = other DNA
  modified_base 5: mod_base = OTHER; note = 5-(N-(1-naphthylmethyl)carboxamide)-2'-deoxyuridine(Nap-dU)
  modified_base 11: mod_base = OTHER; note = 5-(N-(1-naphthylmethyl)carboxamide)-2'-deoxyuridine(Nap-dU)
  modified_base 13: mod_base = OTHER; note = 5-(N-(1-naphthylmethyl)carboxamide)-2'-deoxyuridine(Nap-dU)
  modified_base 19: mod_base = OTHER; note = 5-(N-(1-naphthylmethyl)carboxamide)-2'-deoxyuridine(Nap-dU)
  modified_base 21: mod_base = OTHER; note = 5-(N-(1-naphthylmethyl)carboxamide)-2'-deoxyuridine(Nap-dU)
  modified_base 23: mod_base = OTHER; note = 5-(N-(1-naphthylmethyl)carboxamide)-2'-deoxyuridine(Nap-dU)
caggncgagcngnacgcgngngngacc

SEQ ID NO: 9 - DNA, 74 bp, synthetic construct
  source 1..74: mol_type = other DNA
  misc_binding 1: bound_moiety = Biotin is biding to the 1st residue (5' end)
  misc_difference 17..56: note = The "n" can be replaced with the sequence of each nucleic acid ligand of the nucleic acid ligand library.
gctggtggtgtggctgnnnnnnnnnnnnnnnnnnnnnnnnnnnnnnnnnnnnnnnncaggcagacggtcactca

SEQ ID NO: 10 - DNA, 17 bp, synthetic construct
  source 1..17: mol_type = other DNA
gagtgaccgtctgcctg

SEQ ID NO: 11 - DNA, 16 bp, synthetic construct
  source 1..16: mol_type = other DNA
  misc_binding 1: bound_moiety = Biotin is biding to the 1st residue of the primer (5' end)
gctggtggtgtggctg

SEQ ID NO: 12 - DNA, 16 bp, synthetic construct
  source 1..16: mol_type = other DNA
gctggtggtgtggctg

SEQ ID NO: 13 - DNA, 74 bp, synthetic construct
  source 1..74: mol_type = other DNA
  modified_base 21: mod_base = OTHER; note = 5-(N-(1-naphthylmethyl)carboxamide)-2'-deoxyuridine(Nap-dU)
  modified_base 23: mod_base = OTHER; note = 5-(N-(1-naphthylmethyl)carboxamide)-2'-deoxyuridine(Nap-dU)
  modified_base 25..26: mod_base = OTHER; note = 5-(N-(1-naphthylmethyl)carboxamide)-2'-deoxyuridine(Nap-dU)
  modified_base 30: mod_base = OTHER; note = 5-(N-(1-naphthylmethyl)carboxamide)-2'-deoxyuridine(Nap-dU)
  modified_base 32: mod_base = OTHER; note = 5-(N-(1-naphthylmethyl)carboxamide)-2'-deoxyuridine(Nap-dU)
  modified_base 34: mod_base = OTHER; note = 5-(N-(1-naphthylmethyl)carboxamide)-2'-deoxyuridine(Nap-dU)
  modified_base 40: mod_base = OTHER; note = 5-(N-(1-naphthylmethyl)carboxamide)-2'-deoxyuridine(Nap-dU)
  modified_base 42: mod_base = OTHER; note = 5-(N-(1-naphthylmethyl)carboxamide)-2'-deoxyuridine(Nap-dU)
  modified_base 45: mod_base = OTHER; note = 5-(N-(1-naphthylmethyl)carboxamide)-2'-deoxyuridine(Nap-dU)
  modified_base 48: mod_base = OTHER; note = 5-(N-(1-naphthylmethyl)carboxamide)-2'-deoxyuridine(Nap-dU)
  modified_base 50: mod_base = OTHER; note = 5-(N-(1-naphthylmethyl)carboxamide)-2'-deoxyuridine(Nap-dU)
  modified_base 54: mod_base = OTHER; note = 5-(N-(1-naphthylmethyl)carboxamide)-2'-deoxyuridine(Nap-dU)
gagtgaccgtctgcctggacnangnncgancnancacggncncgngancncganagacagccacaccaccagcc

SEQ ID NO: 14 - DNA, 74 bp, synthetic construct
  source 1..74: mol_type = other DNA
  modified_base 23: mod_base = OTHER; note = 5-(N-(1-naphthylmethyl)carboxamide)-2'-deoxyuridine(Nap-dU)
  modified_base 26: mod_base = OTHER; note = 5-(N-(1-naphthylmethyl)carboxamide)-2'-deoxyuridine(Nap-dU)
  modified_base 28..29: mod_base = OTHER; note = 5-(N-(1-naphthylmethyl)carboxamide)-2'-deoxyuridine(Nap-dU)
  modified_base 35: mod_base = OTHER; note = 5-(N-(1-naphthylmethyl)carboxamide)-2'-deoxyuridine(Nap-dU)
  modified_base 37: mod_base = OTHER; note = 5-(N-(1-naphthylmethyl)carboxamide)-2'-deoxyuridine(Nap-dU)
  modified_base 43..44: mod_base = OTHER; note = 5-(N-(1-naphthylmethyl)carboxamide)-2'-deoxyuridine(Nap-dU)
  modified_base 52: mod_base = OTHER; note = 5-(N-(1-naphthylmethyl)carboxamide)-2'-deoxyuridine(Nap-dU)
  modified_base 55..56: mod_base = OTHER; note = 5-(N-(1-naphthylmethyl)carboxamide)-2'-deoxyuridine(Nap-dU)
gagtgaccgtctgcctgaggccngancnngaaggnanagaacnnaacgcggncgnnacagccacaccaccagcc

SEQ ID NO: 15 - DNA, 74 bp, synthetic construct
  source 1..74: mol_type = other DNA
  modified_base 20: mod_base = OTHER; note = 5-(N-(1-naphthylmethyl)carboxamide)-2'-deoxyuridine(Nap-dU)
  modified_base 24..25: mod_base = OTHER; note = 5-(N-(1-naphthylmethyl)carboxamide)-2'-deoxyuridine(Nap-dU)
  modified_base 27: mod_base = OTHER; note = 5-(N-(1-naphthylmethyl)carboxamide)-2'-deoxyuridine(Nap-dU)
  modified_base 31..33: mod_base = OTHER; note = 5-(N-(1-naphthylmethyl)carboxamide)-2'-deoxyuridine(Nap-dU)
  modified_base 35: mod_base = OTHER; note = 5-(N-(1-naphthylmethyl)carboxamide)-2'-deoxyuridine(Nap-dU)
  modified_base 47: mod_base = OTHER; note = 5-(N-(1-naphthylmethyl)carboxamide)-2'-deoxyuridine(Nap-dU)
  modified_base 49: mod_base = OTHER; note = 5-(N-(1-naphthylmethyl)carboxamide)-2'-deoxyuridine(Nap-dU)
gagtgaccgtctgcctgaanggcnncngccnnngnaacacggcaacngnccacggaccagccacaccaccagcc

SEQ ID NO: 16 - DNA, 74 bp, synthetic construct
  source 1..74: mol_type = other DNA
  modified_base 22..23: mod_base = OTHER; note = 5-(N-(1-naphthylmethyl)carboxamide)-2'-deoxyuridine(Nap-dU)
  modified_base 25: mod_base = OTHER; note = 5-(N-(1-naphthylmethyl)carboxamide)-2'-deoxyuridine(Nap-dU)
  modified_base 29: mod_base = OTHER; note = 5-(N-(1-naphthylmethyl)carboxamide)-2'-deoxyuridine(Nap-dU)
  modified_base 31: mod_base = OTHER; note = 5-(N-(1-naphthylmethyl)carboxamide)-2'-deoxyuridine(Nap-dU)
  modified_base 34: mod_base = OTHER; note = 5-(N-(1-naphthylmethyl)carboxamide)-2'-deoxyuridine(Nap-dU)
  modified_base 39: mod_base = OTHER; note = 5-(N-(1-naphthylmethyl)carboxamide)-2'-deoxyuridine(Nap-dU)
  modified_base 46: mod_base = OTHER; note = 5-(N-(1-naphthylmethyl)carboxamide)-2'-deoxyuridine(Nap-dU)
gagtgaccgtctgcctgccgcnnangagncncgngaganggaccgngcgccagcccccagccacaccaccagcc

SEQ ID NO: 17 - DNA, 72 bp, synthetic construct
  source 1..72: mol_type = other DNA
  modified_base 17: mod_base = OTHER; note = 5-(N-(1-naphthylmethyl)carboxamide)-2'-deoxyuridine(Nap-dU)
  modified_base 20: mod_base = OTHER; note = 5-(N-(1-naphthylmethyl)carboxamide)-2'-deoxyuridine(Nap-dU)
  modified_base 22: mod_base = OTHER; note = 5-(N-(1-naphthylmethyl)carboxamide)-2'-deoxyuridine(Nap-dU)
  modified_base 25: mod_base = OTHER; note = 5-(N-(1-naphthylmethyl)carboxamide)-2'-deoxyuridine(Nap-dU)
  modified_base 28: mod_base = OTHER; note = 5-(N-(1-naphthylmethyl)carboxamide)-2'-deoxyuridine(Nap-dU)
  modified_base 30..31: mod_base = OTHER; note = 5-(N-(1-naphthylmethyl)carboxamide)-2'-deoxyuridine(Nap-dU)
  modified_base 36: mod_base = OTHER; note = 5-(N-(1-naphthylmethyl)carboxamide)-2'-deoxyuridine(Nap-dU)
  modified_base 42..43: mod_base = OTHER; note = 5-(N-(1-naphthylmethyl)carboxamide)-2'-deoxyuridine(Nap-dU)
  modified_base 51: mod_base = OTHER; note = 5-(N-(1-naphthylmethyl)carboxamide)-2'-deoxyuridine(Nap-dU)
  modified_base 54: mod_base = OTHER; note = 5-(N-(1-naphthylmethyl)carboxamide)-2'-deoxyuridine(Nap-dU)
gagtgaccgtctgcctnagngngangancnngacanagaacnnaaccgganggncacagccacaccaccagc

SEQ ID NO: 18 - DNA, 73 bp, synthetic construct
  source 1..73: mol_type = other DNA
  modified_base 19: mod_base = OTHER; note = 5-(N-(1-naphthylmethyl)carboxamide)-2'-deoxyuridine(Nap-dU)
  modified_base 23: mod_base = OTHER; note = 5-(N-(1-naphthylmethyl)carboxamide)-2'-deoxyuridine(Nap-dU)
  modified_base 25: mod_base = OTHER; note = 5-(N-(1-naphthylmethyl)carboxamide)-2'-deoxyuridine(Nap-dU)
  modified_base 27: mod_base = OTHER; note = 5-(N-(1-naphthylmethyl)carboxamide)-2'-deoxyuridine(Nap-dU)
  modified_base 29: mod_base = OTHER; note = 5-(N-(1-naphthylmethyl)carboxamide)-2'-deoxyuridine(Nap-dU)
  modified_base 34: mod_base = OTHER; note = 5-(N-(1-naphthylmethyl)carboxamide)-2'-deoxyuridine(Nap-dU)
  modified_base 37: mod_base = OTHER; note = 5-(N-(1-naphthylmethyl)carboxamide)-2'-deoxyuridine(Nap-dU)
  modified_base 39: mod_base = OTHER; note = 5-(N-(1-naphthylmethyl)carboxamide)-2'-deoxyuridine(Nap-dU)
  modified_base 44: mod_base = OTHER; note = 5-(N-(1-naphthylmethyl)carboxamide)-2'-deoxyuridine(Nap-dU)
  modified_base 46: mod_base = OTHER; note = 5-(N-(1-naphthylmethyl)carboxamide)-2'-deoxyuridine(Nap-dU)
  modified_base 49: mod_base = OTHER; note = 5-(N-(1-naphthylmethyl)carboxamide)-2'-deoxyuridine(Nap-dU)
  modified_base 51: mod_base = OTHER; note = 5-(N-(1-naphthylmethyl)carboxamide)-2'-deoxyuridine(Nap-dU)
  modified_base 54: mod_base = OTHER; note = 5-(N-(1-naphthylmethyl)carboxamide)-2'-deoxyuridine(Nap-dU)
gagtgaccgtctgcctgcngaangncngncaaanacnanacggncncgnancangacagccacaccaccagcc

SEQ ID NO: 19 - DNA, 73 bp, synthetic construct
  source 1..73: mol_type = other DNA
  modified_base 17: mod_base = OTHER; note = 5-(N-(1-naphthylmethyl)carboxamide)-2'-deoxyuridine(Nap-dU)
  modified_base 20: mod_base = OTHER; note = 5-(N-(1-naphthylmethyl)carboxamide)-2'-deoxyuridine(Nap-dU)
  modified_base 25: mod_base = OTHER; note = 5-(N-(1-naphthylmethyl)carboxamide)-2'-deoxyuridine(Nap-dU)
  modified_base 28: mod_base = OTHER; note = 5-(N-(1-naphthylmethyl)carboxamide)-2'-deoxyuridine(Nap-dU)
  modified_base 30..31: mod_base = OTHER; note = 5-(N-(1-naphthylmethyl)carboxamide)-2'-deoxyuridine(Nap-dU)
  modified_base 36: mod_base = OTHER; note = 5-(N-(1-naphthylmethyl)carboxamide)-2'-deoxyuridine(Nap-dU)
  modified_base 42..43: mod_base = OTHER; note = 5-(N-(1-naphthylmethyl)carboxamide)-2'-deoxyuridine(Nap-dU)
  modified_base 51: mod_base = OTHER; note = 5-(N-(1-naphthylmethyl)carboxamide)-2'-deoxyuridine(Nap-dU)
  modified_base 54: mod_base = OTHER; note = 5-(N-(1-naphthylmethyl)carboxamide)-2'-deoxyuridine(Nap-dU)
gagtgaccgtctgcctnagngggangancnngccanagaacnnaaccgganggncacagccacaccaccagcc

SEQ ID NO: 20 - DNA, 73 bp, synthetic construct
  source 1..73: mol_type = other DNA
  modified_base 19: mod_base = OTHER; note = 5-(N-(1-naphthylmethyl)carboxamide)-2'-deoxyuridine(Nap-dU)
  modified_base 23: mod_base = OTHER; note = 5-(N-(1-naphthylmethyl)carboxamide)-2'-deoxyuridine(Nap-dU)
  modified_base 25: mod_base = OTHER; note = 5-(N-(1-naphthylmethyl)carboxamide)-2'-deoxyuridine(Nap-dU)
  modified_base 27: mod_base = OTHER; note = 5-(N-(1-naphthylmethyl)carboxamide)-2'-deoxyuridine(Nap-dU)
  modified_base 29: mod_base = OTHER; note = 5-(N-(1-naphthylmethyl)carboxamide)-2'-deoxyuridine(Nap-dU)
  modified_base 34: mod_base = OTHER; note = 5-(N-(1-naphthylmethyl)carboxamide)-2'-deoxyuridine(Nap-dU)
  modified_base 37: mod_base = OTHER; note = 5-(N-(1-naphthylmethyl)carboxamide)-2'-deoxyuridine(Nap-dU)
  modified_base 39: mod_base = OTHER; note = 5-(N-(1-naphthylmethyl)carboxamide)-2'-deoxyuridine(Nap-dU)
  modified_base 44: mod_base = OTHER; note = 5-(N-(1-naphthylmethyl)carboxamide)-2'-deoxyuridine(Nap-dU)
  modified_base 46: mod_base = OTHER; note = 5-(N-(1-naphthylmethyl)carboxamide)-2'-deoxyuridine(Nap-dU)
  modified_base 49: mod_base = OTHER; note = 5-(N-(1-naphthylmethyl)carboxamide)-2'-deoxyuridine(Nap-dU)
  modified_base 51: mod_base = OTHER; note = 5-(N-(1-naphthylmethyl)carboxamide)-2'-deoxyuridine(Nap-dU)
  modified_base 54: mod_base = OTHER; note = 5-(N-(1-naphthylmethyl)carboxamide)-2'-deoxyuridine(Nap-dU)
gagtgaccgtctgcctacnaaangncngncaaanacnanacggncncgnancangacagccacaccaccagcc

SEQ ID NO: 21 - DNA, 71 bp, synthetic construct
  source 1..71: mol_type = other DNA
  modified_base 17: mod_base = OTHER; note = Nucleic acid ligand(Full length) derived from Clone 1
  modified_base 19..20: mod_base = OTHER; note = Nucleic acid ligand(Full length) derived from Clone 1
  modified_base 25: mod_base = OTHER; note = Nucleic acid ligand(Full length) derived from Clone 1
  modified_base 31..32: mod_base = OTHER; note = Nucleic acid ligand(Full length) derived from Clone 1
  modified_base 39: mod_base = OTHER; note = Nucleic acid ligand(Full length) derived from Clone 1
  modified_base 41: mod_base = OTHER; note = Nucleic acid ligand(Full length) derived from Clone 1
  modified_base 44..45: mod_base = OTHER; note = Nucleic acid ligand(Full length) derived from Clone 1
  modified_base 53: mod_base = OTHER; note = Nucleic acid ligand(Full length) derived from Clone 1
gagtgaccgtctgcctncnngaacnagaacnnaaccgcnanggnnacagcggnacagccacaccaccagcc

SEQ ID NO: 22 - DNA, 73 bp, synthetic construct
  source 1..73: mol_type = other DNA
  modified_base 17: mod_base = OTHER; note = 5-(N-(1-naphthylmethyl)carboxamide)-2'-deoxyuridine(Nap-dU)
  modified_base 20: mod_base = OTHER; note = 5-(N-(1-naphthylmethyl)carboxamide)-2'-deoxyuridine(Nap-dU)
  modified_base 25: mod_base = OTHER; note = 5-(N-(1-naphthylmethyl)carboxamide)-2'-deoxyuridine(Nap-dU)
  modified_base 28: mod_base = OTHER; note = 5-(N-(1-naphthylmethyl)carboxamide)-2'-deoxyuridine(Nap-dU)
  modified_base 30..31: mod_base = OTHER; note = 5-(N-(1-naphthylmethyl)carboxamide)-2'-deoxyuridine(Nap-dU)
  modified_base 36: mod_base = OTHER; note = 5-(N-(1-naphthylmethyl)carboxamide)-2'-deoxyuridine(Nap-dU)
  modified_base 42..44: mod_base = OTHER; note = 5-(N-(1-naphthylmethyl)carboxamide)-2'-deoxyuridine(Nap-dU)
  modified_base 51: mod_base = OTHER; note = 5-(N-(1-naphthylmethyl)carboxamide)-2'-deoxyuridine(Nap-dU)
  modified_base 54..55: mod_base = OTHER; note = 5-(N-(1-naphthylmethyl)carboxamide)-2'-deoxyuridine(Nap-dU)
gagtgaccgtctgcctnagngggangancnngcaanagaacnnnaccgganggnnacagccacaccaccagcc

SEQ ID NO: 23 - DNA, 40 bp, synthetic construct
  source 1..40: mol_type = other DNA
  modified_base 2: mod_base = OTHER; note = 5-(N-(1-naphthylmethyl)carboxamide)-2'-deoxyuridine(Nap-dU)
  modified_base 4..5: mod_base = OTHER; note = 5-(N-(1-naphthylmethyl)carboxamide)-2'-deoxyuridine(Nap-dU)
  modified_base 10..12: mod_base = OTHER; note = 5-(N-(1-naphthylmethyl)carboxamide)-2'-deoxyuridine(Nap-dU)
  modified_base 16: mod_base = OTHER; note = 5-(N-(1-naphthylmethyl)carboxamide)-2'-deoxyuridine(Nap-dU)
  modified_base 20: mod_base = OTHER; note = 5-(N-(1-naphthylmethyl)carboxamide)-2'-deoxyuridine(Nap-dU)
  modified_base 24: mod_base = OTHER; note = 5-(N-(1-naphthylmethyl)carboxamide)-2'-deoxyuridine(Nap-dU)
  modified_base 35: mod_base = OTHER; note = 5-(N-(1-naphthylmethyl)carboxamide)-2'-deoxyuridine(Nap-dU)
angnnagagnnngccngagngccncgcaagggcgnaacaa